European Patent Application EP 4 556 494 A1, published May 21, 2025. Title: ANTI-ROR1 ANTIBODY, BISPECIFIC ANTIBODY COMPRISING THE SAME, AND USES THEREOF. Applicant: ABL Bio Inc. The sequence listing filed with the application follows.

SEQUENCE LISTING (127 sequences)

SEQ ID NO: 1 - protein, 5 aa, synthetic construct
  REGION 1..5: note = HCDR1_anti-ROR1 antibody
NYDMS

SEQ ID NO: 2 - protein, 17 aa, synthetic construct
  REGION 1..17: note = HCDR2_anti-ROR1 antibody
AIYHSGSSKYYADSVKG

SEQ ID NO: 3 - protein, 12 aa, synthetic construct
  REGION 1..12: note = HCDR3_anti-ROR1 antibody
GGSGAWDTGFDY

SEQ ID NO: 4 - protein, 13 aa, synthetic construct
  REGION 1..13: note = LCDR1_anti-ROR1 antibody
SGSSSNIGSNDVS

SEQ ID NO: 5 - protein, 7 aa, synthetic construct
  REGION 1..7: note = LCDR2_anti-ROR1 antibody
YENNRPS

SEQ ID NO: 6 - protein, 11 aa, synthetic construct
  REGION 1..11: note = LCDR3_anti-ROR1 antibody
GAWDDSLSGYV

SEQ ID NO: 7 - protein, 121 aa, synthetic construct
  REGION 1..121: note = heavy chain variable region_anti-ROR1 antibody (IgG)
EVQLLESGGGLVQPGGSLRLSCAASGFTFSNYDMSWVRQAPGKGLEWVSAIYHSGSSKYYADSVKGRFTISRDNSKNTLYLQMNSLRAEDTAVYYCARGGSGAWDTGFDYWGQGTLVTVSS

SEQ ID NO: 8 - protein, 110 aa, synthetic construct
  REGION 1..110: note = light chain variable region_anti-ROR1 antibody (IgG)
QSVLTQPPSASGTPGQRVTISCSGSSSNIGSNDVSWYQQLPGTAPKLLIYYENNRPSGVPDRFSGSKSGTSASLAISGLRSEDEADYYCGAWDDSLSGYVFGGGTKLTVL

SEQ ID NO: 9 - protein, 12 aa, synthetic construct
  REGION 1..12: note = HCDR3_anti-ROR1 antibody
GGNGAWDTGFDY

SEQ ID NO: 10 - protein, 7 aa, synthetic construct
  REGION 1..7: note = LCDR2_anti-ROR1 antibody
YDNNRPS

SEQ ID NO: 11 - protein, 121 aa, synthetic construct
  REGION 1..121: note = heavy chain variable region_anti-ROR1 antibody
EVQLLESGGGLVQPGGSLRLSCAASGFTFSNYDMSWVRQAPGKGLEWVSAIYHSGSSKYYADSVKGRFTISRDNSKNTLYLQMNSLRAEDTAVYYCARGGNGAWDTGFDYWGQGTLVTVSS

SEQ ID NO: 12 - protein, 110 aa, synthetic construct
  REGION 1..110: note = light chain variable region_anti-ROR1 antibody
QSVLTQPPSASGTPGQRVTISCSGSSSNIGSNDVSWYQQLPGTAPKLLIYYDNNRPSGVPDRFSGSKSGTSASLAISGLRSEDEADYYCGAWDDSLSGYVFGGGTKLTVL

SEQ ID NO: 13 - protein, 5 aa, synthetic construct
  REGION 1..5: note = HCDR1_anti-4-1BB antibody
SYDMS

SEQ ID NO: 14 - protein, 5 aa, synthetic construct
  REGION 1..5: note = HCDR1_anti-4-1BB antibody
GYDMS

SEQ ID NO: 15 - protein, 5 aa, synthetic construct
  REGION 1..5: note = HCDR1_anti-4-1BB antibody
SYWMH

SEQ ID NO: 16 - protein, 17 aa, synthetic construct
  REGION 1..17: note = HCDR2_anti-4-1BB antibody
WISYSGGSIYYADSVKG

SEQ ID NO: 17 - protein, 17 aa, synthetic construct
  REGION 1..17: note = HCDR2_anti-4-1BB antibody
VIYPDDGNTYYADSVKG

SEQ ID NO: 18 - protein, 17 aa, synthetic construct
  REGION 1..17: note = HCDR2_anti-4-1BB antibody
EINPGNGHTNYNEKFKS

SEQ ID NO: 19 - protein, 12 aa, synthetic construct
  REGION 1..12: note = HCDR3_anti-4-1BB antibody
DGQRNSMREFDY

SEQ ID NO: 20 - protein, 12 aa, synthetic construct
  REGION 1..12: note = HCDR3_anti-4-1BB antibody
DAQRNSMREFDY

SEQ ID NO: 21 - protein, 12 aa, synthetic construct
  REGION 1..12: note = HCDR3_anti-4-1BB antibody
DAQRQSMREFDY

SEQ ID NO: 22 - protein, 18 aa, synthetic construct
  REGION 1..18: note = HCDR3_anti-4-1BB antibody
HGGQKPTTKSSSAYGMDG

SEQ ID NO: 23 - protein, 10 aa, synthetic construct
  REGION 1..10: note = HCDR3_anti-4-1BB antibody
SFTTARAFAY

SEQ ID NO: 24 - protein, 13 aa, synthetic construct
  REGION 1..13: note = LCDR1_anti-4-1BB antibody
SGSSSNIGNNYVT

SEQ ID NO: 25 - protein, 11 aa, synthetic construct
  REGION 1..11: note = LCDR1_anti-4-1BB antibody
RASQTISDYLH

SEQ ID NO: 26 - protein, 7 aa, synthetic construct
  REGION 1..7: note = LCDR2_anti-4-1BB antibody
ADSHRPS

SEQ ID NO: 27 - protein, 7 aa, synthetic construct
  REGION 1..7: note = LCDR2_anti-4-1BB antibody
YASQSIS

SEQ ID NO: 28 - protein, 11 aa, synthetic construct
  REGION 1..11: note = LCDR3_anti-4-1BB antibody
ATWDYSLSGYV

SEQ ID NO: 29 - protein, 9 aa, synthetic construct
  REGION 1..9: note = LCDR3_anti-4-1BB antibody
QDGHSFPPT

SEQ ID NO: 30 - protein, 121 aa, synthetic construct
  REGION 1..121: note = heavy chain variable region_anti-4-1BB antibody
EVQLLESGGGLVQPGGSLRLSCAASGFTFSSYDMSWVRQAPGKGLEWVSWISYSGGSIYYADSVKGRFTISRDNSKNTLYLQMNSLRAEDTAVYYCARDGQRNSMREFDYWGQGTLVTVSS

SEQ ID NO: 31 - protein, 121 aa, synthetic construct
  REGION 1..121: note = heavy chain variable region_anti-4-1BB antibody
EVQLLESGGGLVQPGGSLRLSCAASGFTFSSYDMSWVRQAPGKGLEWVSWISYSGGSIYYADSVKGRFTISRDNSKNTLYLQMNSLRAEDTAVYYCARDAQRNSMREFDYWGQGTLVTVSS

SEQ ID NO: 32 - protein, 121 aa, synthetic construct
  REGION 1..121: note = heavy chain variable region_anti-4-1BB antibody
EVQLLESGGGLVQPGGSLRLSCAASGFTFSSYDMSWVRQAPGKGLEWVSWISYSGGSIYYADSVKGRFTISRDNSKNTLYLQMNSLRAEDTAVYYCARDAQRQSMREFDYWGQGTLVTVSS

SEQ ID NO: 33 - protein, 127 aa, synthetic construct
  REGION 1..127: note = heavy chain variable region_anti-4-1BB antibody
EVQLLESGGGLVQPGGSLRLSCAASGFTFSGYDMSWVRQAPGKGLEWVSVIYPDDGNTYYADSVKGRFTISRDNSKNTLYLQMNSLRAEDAAVYYCAKHGGQKPTTKSSSAYGMDGWGQGTLVTVSS

SEQ ID NO: 34 - protein, 127 aa, synthetic construct
  REGION 1..127: note = heavy chain variable region_anti-4-1BB antibody
EVQLLESGGGLVQPGGSLRLSCAASGFTFSGYDMSWVRQAPGKGLEWVSVIYPDDGNTYYADSVKGRFTISRDNSKNTLYLQMNSLRAEDTAVYYCAKHGGQKPTTKSSSAYGMDGWGQGTLVTVSS

SEQ ID NO: 35 - protein, 119 aa, synthetic construct
  REGION 1..119: note = heavy chain variable region_anti-4-1BB antibody
QVQLQQSGAEVIKPGASVKLSCKASGYTFSSYWMHWVRQAPGQGLEWIGEINPGNGHTNYNEKFKSRATLTGDTSTSTVYMELSSLRSEDTAVYYCARSFTTARAFAYWGQGTLVTVSS

SEQ ID NO: 36 - protein, 121 aa, synthetic construct
  REGION 1..121: note = heavy chain variable region_anti-4-1BB antibody
EVQLLESGGGLVQPGGSLRLSCAASGFTFSSYDMSWVRQAPGKCLEWVSWISYSGGSIYYADSVKGRFTISRDNSKNTLYLQMNSLRAEDTAVYYCARDGQRNSMREFDYWGQGTLVTVSS

SEQ ID NO: 37 - protein, 121 aa, synthetic construct
  REGION 1..121: note = heavy chain variable region_anti-4-1BB antibody
EVQLLESGGGLVQPGGSLRLSCAASGFTFSSYDMSWVRQAPGKCLEWVSWISYSGGSIYYADSVKGRFTISRDNSKNTLYLQMNSLRAEDTAVYYCARDAQRNSMREFDYWGQGTLVTVSS

SEQ ID NO: 38 - protein, 121 aa, synthetic construct
  REGION 1..121: note = heavy chain variable region_anti-4-1BB antibody
EVQLLESGGGLVQPGGSLRLSCAASGFTFSSYDMSWVRQAPGKCLEWVSWISYSGGSIYYADSVKGRFTISRDNSKNTLYLQMNSLRAEDTAVYYCARDAQRQSMREFDYWGQGTLVTVSS

SEQ ID NO: 39 - protein, 127 aa, synthetic construct
  REGION 1..127: note = heavy chain variable region_anti-4-1BB antibody
EVQLLESGGGLVQPGGSLRLSCAASGFTFSGYDMSWVRQAPGKCLEWVSVIYPDDGNTYYADSVKGRFTISRDNSKNTLYLQMNSLRAEDAAVYYCAKHGGQKPTTKSSSAYGMDGWGQGTLVTVSS

SEQ ID NO: 40 - protein, 127 aa, synthetic construct
  REGION 1..127: note = heavy chain variable region_anti-4-1BB antibody
EVQLLESGGGLVQPGGSLRLSCAASGFTFSGYDMSWVRQAPGKCLEWVSVIYPDDGNTYYADSVKGRFTISRDNSKNTLYLQMNSLRAEDTAVYYCAKHGGQKPTTKSSSAYGMDGWGQGTLVTVSS

SEQ ID NO: 41 - protein, 119 aa, synthetic construct
  REGION 1..119: note = heavy chain variable region_anti-4-1BB antibody
QVQLQQSGAEVIKPGASVKLSCKASGYTFSSYWMHWVRQAPGQCLEWIGEINPGNGHTNYNEKFKSRATLTGDTSTSTVYMELSSLRSEDTAVYYCARSFTTARAFAYWGQGTLVTVSS

SEQ ID NO: 42 - protein, 110 aa, synthetic construct
  REGION 1..110: note = light chain variable region_anti-4-1BB antibody
QSVLTQPPSASGTPGRRVTISCSGSSSNIGNNYVTWYQQLPGTAPKLLIYADSHRPSGVPDRFSGSKSGTSASLAISGLRSEDEADYYCATWDYSLSGYVFGGGTKLTVL

SEQ ID NO: 43 - protein, 110 aa, synthetic construct
  REGION 1..110: note = light chain variable region_anti-4-1BB antibody
QSVLTQPPSASGTPGQRVTISCSGSSSNIGNNYVTWYQQLPGTAPKLLIYADSHRPSGVPDRFSGSKSGTSASLAISGLRSEDEADYYCATWDYSLSGYVFGGGTKLTVL

SEQ ID NO: 44 - protein, 108 aa, synthetic construct
  REGION 1..108: note = light chain variable region_anti-4-1BB antibody
DIVMTQSPAFLSVTPGEKVTITCRASQTISDYLHWYQQKPDQAPKLLIKYASQSISGIPSRFSGSGSGTDFTFTISSLEAEDAATYYCQDGHSFPPTFGQGTKLEIKR

SEQ ID NO: 45 - protein, 110 aa, synthetic construct
  REGION 1..110: note = light chain variable region_anti-4-1BB antibody
QSVLTQPPSASGTPGRRVTISCSGSSSNIGNNYVTWYQQLPGTAPKLLIYADSHRPSGVPDRFSGSKSGTSASLAISGLRSEDEADYYCATWDYSLSGYVFGCGTKLTVL

SEQ ID NO: 46 - protein, 110 aa, synthetic construct
  REGION 1..110: note = light chain variable region_anti-4-1BB antibody
QSVLTQPPSASGTPGQRVTISCSGSSSNIGNNYVTWYQQLPGTAPKLLIYADSHRPSGVPDRFSGSKSGTSASLAISGLRSEDEADYYCATWDYSLSGYVFGCGTKLTVL

SEQ ID NO: 47 - protein, 108 aa, synthetic construct
  REGION 1..108: note = light chain variable region_anti-4-1BB antibody
DIVMTQSPAFLSVTPGEKVTITCRASQTISDYLHWYQQKPDQAPKLLIKYASQSISGIPSRFSGSGSGTDFTFTISSLEAEDAATYYCQDGHSFPPTFGCGTKLEIKR

SEQ ID NO: 48 - protein, 5 aa, synthetic construct
  REGION 1..5: note = HCDR1_anti-B7-H3 antibody
DYAMS

SEQ ID NO: 49 - protein, 5 aa, synthetic construct
  REGION 1..5: note = HCDR1_anti-B7-H3 antibody
GYYMS

SEQ ID NO: 50 - protein, 5 aa, synthetic construct
  REGION 1..5: note = HCDR1_anti-B7-H3 antibody
SYSMS

SEQ ID NO: 51 - protein, 5 aa, synthetic construct
  REGION 1..5: note = HCDR1_anti-B7-H3 antibody
SYGMS

SEQ ID NO: 52 - protein, 17 aa, synthetic construct
  REGION 1..17: note = HCDR2_anti-B7-H3 antibody
SISSGSGSIYYADSVKG

SEQ ID NO: 53 - protein, 17 aa, synthetic construct
  REGION 1..17: note = HCDR2_anti-B7-H3 antibody
LISPSSGSIYYADSVKG

SEQ ID NO: 54 - protein, 17 aa, synthetic construct
  REGION 1..17: note = HCDR2_anti-B7-H3 antibody
GIYSDGSNTYYADSVKG

SEQ ID NO: 55 - protein, 17 aa, synthetic construct
  REGION 1..17: note = HCDR2_anti-B7-H3 antibody
GISPGGSNTYYADSVKG

SEQ ID NO: 56 - protein, 17 aa, synthetic construct
  REGION 1..17: note = HCDR2_anti-B7-H3 antibody
GIYSGGSSKYYADSVKG

SEQ ID NO: 57 - protein, 17 aa, synthetic construct
  REGION 1..17: note = HCDR2_anti-B7-H3 antibody
GIYSDASNTYYADSVKG

SEQ ID NO: 58 - protein, 7 aa, synthetic construct
  REGION 1..7: note = HCDR3_anti-B7-H3 antibody
NLIPLDY

SEQ ID NO: 59 - protein, 7 aa, synthetic construct
  REGION 1..7: note = HCDR3_anti-B7-H3 antibody
GLTKFDY

SEQ ID NO: 60 - protein, 7 aa, synthetic construct
  REGION 1..7: note = HCDR3_anti-B7-H3 antibody
MLHRFDY

SEQ ID NO: 61 - protein, 12 aa, synthetic construct
  REGION 1..12: note = HCDR3_anti-B7-H3 antibody
DAWIARLLLFDY

SEQ ID NO: 62 - protein, 7 aa, synthetic construct
  REGION 1..7: note = HCDR3_anti-B7-H3 antibody
NRLRFDY

SEQ ID NO: 63 - protein, 13 aa, synthetic construct
  REGION 1..13: note = LCDR1_anti-B7-H3 antibody
SGSSSNIGSNAVS

SEQ ID NO: 64 - protein, 13 aa, synthetic construct
  REGION 1..13: note = LCDR1_anti-B7-H3 antibody
TGSSSNIGSNDVS

SEQ ID NO: 65 - protein, 13 aa, synthetic construct
  REGION 1..13: note = LCDR1_anti-B7-H3 antibody
SGSSSNIGSNSVT

SEQ ID NO: 66 - protein, 13 aa, synthetic construct
  REGION 1..13: note = LCDR1_anti-B7-H3 antibody
SGSSSNIGSNAVT

SEQ ID NO: 67 - protein, 13 aa, synthetic construct
  REGION 1..13: note = LCDR1_anti-B7-H3 antibody
TGSSSNIGSNSVT

SEQ ID NO: 68 - protein, 7 aa, synthetic construct
  REGION 1..7: note = LCDR2_anti-B7-H3 antibody
YNSHRPS

SEQ ID NO: 69 - protein, 7 aa, synthetic construct
  REGION 1..7: note = LCDR2_anti-B7-H3 antibody
ANSHRPS

SEQ ID NO: 70 - protein, 7 aa, synthetic construct
  REGION 1..7: note = LCDR2_anti-B7-H3 antibody
ADSQRPS

SEQ ID NO: 71 - protein, 7 aa, synthetic construct
  REGION 1..7: note = LCDR2_anti-B7-H3 antibody
YNNKRPS

SEQ ID NO: 72 - protein, 7 aa, synthetic construct
  REGION 1..7: note = LCDR2_anti-B7-H3 antibody
SDSHRPS

SEQ ID NO: 73 - protein, 7 aa, synthetic construct
  REGION 1..7: note = LCDR2_anti-B7-H3 antibody
ADVQRPS

SEQ ID NO: 74 - protein, 11 aa, synthetic construct
  REGION 1..11: note = LCDR3_anti-B7-H3 antibody
GSWDASLNAYV

SEQ ID NO: 75 - protein, 11 aa, synthetic construct
  REGION 1..11: note = LCDR3_anti-B7-H3 antibody
GSWDDSLSGYV

SEQ ID NO: 76 - protein, 11 aa, synthetic construct
  REGION 1..11: note = LCDR3_anti-B7-H3 antibody
GTWDSSLNAYV

SEQ ID NO: 77 - protein, 11 aa, synthetic construct
  REGION 1..11: note = LCDR3_anti-B7-H3 antibody
GTWDDSLSGYV

SEQ ID NO: 78 - protein, 11 aa, synthetic construct
  REGION 1..11: note = LCDR3_anti-B7-H3 antibody
GTWDASLNAYV

SEQ ID NO: 79 - protein, 11 aa, synthetic construct
  REGION 1..11: note = LCDR3_anti-B7-H3 antibody
GSWDASLNAYV

SEQ ID NO: 80 - protein, 116 aa, synthetic construct
  REGION 1..116: note = heavy chain variable region_anti-B7-H3 antibody
EVQLLESGGGLVQPGGSLRLSCAASGFTFSDYAMSWVRQAPGKGLEWVSSISSGSGSIYYADSVKGRFTISRDNSKNTLYLQMNSLRAEDTAVYYCAKNLIPLDYWGQGTLVTVSS

SEQ ID NO: 81 - protein, 116 aa, synthetic construct
  REGION 1..116: note = heavy chain variable region_anti-B7-H3 antibody
EVQLLESGGGLVQPGGSLRLSCAASGFTFSGYYMSWVRQAPGKGLEWVSLISPSSGSIYYADSVKGRFTISRDNSKNTLYLQMNSLRAEDTAVYYCAKGLTKFDYWGQGTLVTVSS

SEQ ID NO: 82 - protein, 116 aa, synthetic construct
  REGION 1..116: note = heavy chain variable region_anti-B7-H3 antibody
EVQLLESGGGLVQPGGSLRLSCAASGFTFSSYSMSWVRQAPGKGLEWVSGIYSDGSNTYYADSVKGRFTISRDNSKNTLYLQMNSLRAEDTAVYYCAKMLHRFDYWGQGTLVTVSS

SEQ ID NO: 83 - protein, 121 aa, synthetic construct
  REGION 1..121: note = heavy chain variable region_anti-B7-H3 antibody
EVQLLESGGGLVQPGGSLRLSCAASGFTFSDYAMSWVRQAPGKGLEWVSGISPGGSNTYYADSVKGRFTISRDNSKNTLYLQMNSLRAEDTAVYYCAKDAWIARLLLFDYWGQGTLVTVSS

SEQ ID NO: 84 - protein, 116 aa, synthetic construct
  REGION 1..116: note = heavy chain variable region_anti-B7-H3 antibody
EVQLLESGGGLVQPGGSLRLSCAASGFTFSSYGMSWVRQAPGKGLEWVSGIYSGGSSKYYADSVKGRFTISRDNSKNTLYLQMNSLRAEDTAVYYCAKNRLRFDYWGQGTLVTVSS

SEQ ID NO: 85 - protein, 116 aa, synthetic construct
  REGION 1..116: note = heavy chain variable region_anti-B7-H3 antibody
EVQLLESGGGLVQPGGSLRLSCAASGFTFSSYSMSWVRQAPGKGLEWVSGIYSDASNTYYADSVKGRFTISRDNSKNTLYLQMNSLRAEDTAVYYCAKMLHRFDYWGQGTLVTVSS

SEQ ID NO: 86 - protein, 116 aa, synthetic construct
  REGION 1..116: note = heavy chain variable region_anti-B7-H3 antibody
EVQLLESGGGLVQPGGSLRLSCAASGFTFSDYAMSWVRQAPGKCLEWVSSISSGSGSIYYADSVKGRFTISRDNSKNTLYLQMNSLRAEDTAVYYCAKNLIPLDYWGQGTLVTVSS

SEQ ID NO: 87 - protein, 116 aa, synthetic construct
  REGION 1..116: note = heavy chain variable region_anti-B7-H3 antibody
EVQLLESGGGLVQPGGSLRLSCAASGFTFSGYYMSWVRQAPGKCLEWVSLISPSSGSIYYADSVKGRFTISRDNSKNTLYLQMNSLRAEDTAVYYCAKGLTKFDYWGQGTLVTVSS

SEQ ID NO: 88 - protein, 116 aa, synthetic construct
  REGION 1..116: note = heavy chain variable region_anti-B7-H3 antibody
EVQLLESGGGLVQPGGSLRLSCAASGFTFSSYSMSWVRQAPGKCLEWVSGIYSDGSNTYYADSVKGRFTISRDNSKNTLYLQMNSLRAEDTAVYYCAKMLHRFDYWGQGTLVTVSS

SEQ ID NO: 89 - protein, 121 aa, synthetic construct
  REGION 1..121: note = heavy chain variable region_anti-B7-H3 antibody
EVQLLESGGGLVQPGGSLRLSCAASGFTFSDYAMSWVRQAPGKCLEWVSGISPGGSNTYYADSVKGRFTISRDNSKNTLYLQMNSLRAEDTAVYYCAKDAWIARLLLFDYWGQGTLVTVSS

SEQ ID NO: 90 - protein, 116 aa, synthetic construct
  REGION 1..116: note = heavy chain variable region_anti-B7-H3 antibody
EVQLLESGGGLVQPGGSLRLSCAASGFTFSSYGMSWVRQAPGKCLEWVSGIYSGGSSKYYADSVKGRFTISRDNSKNTLYLQMNSLRAEDTAVYYCAKNRLRFDYWGQGTLVTVSS

SEQ ID NO: 91 - protein, 116 aa, synthetic construct
  REGION 1..116: note = heavy chain variable region_anti-B7-H3 antibody
EVQLLESGGGLVQPGGSLRLSCAASGFTFSSYSMSWVRQAPGKCLEWVSGIYSDASNTYYADSVKGRFTISRDNSKNTLYLQMNSLRAEDTAVYYCAKMLHRFDYWGQGTLVTVSS

SEQ ID NO: 92 - protein, 110 aa, synthetic construct
  REGION 1..110: note = light chain variable region_anti-B7-H3 antibody
QSVLTQPPSASGTPGQRVTISCSGSSSNIGSNAVSWYQQLPGTAPKLLIYYNSHRPSGVPDRFSGSKSGTSASLAISGLRSEDEADYYCGSWDASLNAYVFGGGTKLTVL

SEQ ID NO: 93 - protein, 110 aa, synthetic construct
  REGION 1..110: note = light chain variable region_anti-B7-H3 antibody
QSVLTQPPSASGTPGQRVTISCTGSSSNIGSNDVSWYQQLPGTAPKLLIYANSHRPSGVPDRFSGSKSGTSASLAISGLRSEDEADYYCGSWDDSLSGYVFGGGTKLTVL

SEQ ID NO: 94 - protein, 110 aa, synthetic construct
  REGION 1..110: note = light chain variable region_anti-B7-H3 antibody
QSVLTQPPSASGTPGQRVTISCSGSSSNIGSNSVTWYQQLPGTAPKLLIYADSQRPSGVPDRFSGSKSGTSASLAISGLRSEDEADYYCGTWDSSLNAYVFGGGTKLTVL

SEQ ID NO: 95 - protein, 110 aa, synthetic construct
  REGION 1..110: note = light chain variable region_anti-B7-H3 antibody
QSVLTQPPSASGTPGQRVTISCSGSSSNIGSNAVTWYQQLPGTAPKLLIYYNNKRPSGVPDRFSGSKSGTSASLAISGLRSEDEADYYCGTWDDSLSGYVFGGGTKLTVL

SEQ ID NO: 96 - protein, 110 aa, synthetic construct
  REGION 1..110: note = light chain variable region_anti-B7-H3 antibody
QSVLTQPPSASGTPGQRVTISCTGSSSNIGSNSVTWYQQLPGTAPKLLIYSDSHRPSGVPDRFSGSKSGTSASLAISGLRSEDEADYYCGTWDASLNAYVFGGGTKLTVL

SEQ ID NO: 97 - protein, 110 aa, synthetic construct
  REGION 1..110: note = light chain variable region_anti-B7-H3 antibody
QSVLTQPPSASGTPGQRVTISCSGSSSNIGSNSVTWYQQLPGTAPKLLIYADVQRPSGVPDRFSGSKSGTSASLAISGLRSEDEADYYCGTWDSSLNAYVFGGGTKLTVL

SEQ ID NO: 98 - protein, 110 aa, synthetic construct
  REGION 1..110: note = light chain variable region_anti-B7-H3 antibody
QSVLTQPPSASGTPGQRVTISCSGSSSNIGSNAVSWYQQLPGTAPKLLIYYNSHRPSGVPDRFSGSKSGTSASLAISGLRSEDEADYYCGSWDASLNAYVFGCGTKLTVL

SEQ ID NO: 99 - protein, 110 aa, synthetic construct
  REGION 1..110: note = light chain variable region_anti-B7-H3 antibody
QSVLTQPPSASGTPGQRVTISCTGSSSNIGSNDVSWYQQLPGTAPKLLIYANSHRPSGVPDRFSGSKSGTSASLAISGLRSEDEADYYCGSWDDSLSGYVFGCGTKLTVL

SEQ ID NO: 100 - protein, 110 aa, synthetic construct
  REGION 1..110: note = light chain variable region_anti-B7-H3 antibody
QSVLTQPPSASGTPGQRVTISCSGSSSNIGSNSVTWYQQLPGTAPKLLIYADSQRPSGVPDRFSGSKSGTSASLAISGLRSEDEADYYCGTWDSSLNAYVFGCGTKLTVL

SEQ ID NO: 101 - protein, 110 aa, synthetic construct
  REGION 1..110: note = light chain variable region_anti-B7-H3 antibody
QSVLTQPPSASGTPGQRVTISCSGSSSNIGSNAVTWYQQLPGTAPKLLIYYNNKRPSGVPDRFSGSKSGTSASLAISGLRSEDEADYYCGTWDDSLSGYVFGCGTKLTVL

SEQ ID NO: 102 - protein, 110 aa, synthetic construct
  REGION 1..110: note = light chain variable region_anti-B7-H3 antibody
QSVLTQPPSASGTPGQRVTISCTGSSSNIGSNSVTWYQQLPGTAPKLLIYSDSHRPSGVPDRFSGSKSGTSASLAISGLRSEDEADYYCGTWDASLNAYVFGCGTKLTVL

SEQ ID NO: 103 - protein, 110 aa, synthetic construct
  REGION 1..110: note = light chain variable region_anti-B7-H3 antibody
QSVLTQPPSASGTPGQRVTISCSGSSSNIGSNSVTWYQQLPGTAPKLLIYADVQRPSGVPDRFSGSKSGTSASLAISGLRSEDEADYYCGTWDSSLNAYVFGCGTKLTVL

SEQ ID NO: 104 - protein, 330 aa, synthetic construct
  REGION 1..330: note = heavy chain constant region(WT)
ASTKGPSVFPLAPSSKSTSGGTAALGCLVKDYFPEPVTVSWNSGALTSGVHTFPAVLQSSGLYSLSSVVTVPSSSLGTQTYICNVNHKPSNTKVDKKVEPKSCDKTHTCPPCPAPELLGGPSVFLFPPKPKDTLMISRTPEVTCVVVDVSHEDPEVKFNWYVDGVEVHNAKTKPREEQYNSTYRVVSVLTVLHQDWLNGKEYKCKVSNKALPAPIEKTISKAKGQPREPQVYTLPPSREEMTKNQVSLTCLVKGFYPSDIAVEWESNGQPENNYKTTPPVLDSDGSFFLYSKLTVDKSRWQQGNVFSCSVMHEALHNHYTQKSLSLSPGK

SEQ ID NO: 105 - protein, 330 aa, synthetic construct
  REGION 1..330: note = Heavy Chain constant region(NA)
ASTKGPSVFPLAPSSKSTSGGTAALGCLVKDYFPEPVTVSWNSGALTSGVHTFPAVLQSSGLYSLSSVVTVPSSSLGTQTYICNVNHKPSNTKVDKKVEPKSCDKTHTCPPCPAPELLGGPSVFLFPPKPKDTLMISRTPEVTCVVVDVSHEDPEVKFNWYVDGVEVHNAKTKPREEQYASTYRVVSVLTVLHQDWLNGKEYKCKVSNKALPAPIEKTISKAKGQPREPQVYTLPPSREEMTKNQVSLTCLVKGFYPSDIAVEWESNGQPENNYKTTPPVLDSDGSFFLYSKLTVDKSRWQQGNVFSCSVMHEALHNHYTQKSLSLSPGK

SEQ ID NO: 106 - DNA, 363 bp, synthetic construct
  misc_feature 1..363: note = DNA encoding heavy chain variable region_BA6M11
  source 1..363: mol_type = other DNA
gaggtgcagctgctggagtccggcggcggcctggtgcagcccggcggctccctgcggctgtcctgcgccgcctccggcttcaccttctccaactacgacatgtcctgggtgcggcaggcccccggcaagggcctggagtgggtgtccgccatctaccactccggctcctccaagtactacgccgactccgtgaagggccggttcaccatctcccgggacaactccaagaacaccctgtacctgcagatgaactccctgcgggccgaggacaccgccgtgtactactgcgcccggggcggctccggcgcctgggacaccggcttcgactactggggccagggcaccctggtgaccgtgtcctcc

SEQ ID NO: 107 - DNA, 990 bp, synthetic construct
  misc_feature 1..990: note = DNA encoding heavy chain constant region (WT)_BA6M11
  source 1..990: mol_type = other DNA
gcctccaccaagggcccctccgtgttccccctggccccctcctccaagtccacctccggcggcaccgccgccctgggctgcctggtgaaggactacttccccgagcccgtgaccgtgtcctggaactccggcgccctgacctccggcgtgcacaccttccccgccgtgctgcagtcctccggcctgtactccctgtcctccgtcgtgaccgtgccctcctcctccctgggcacccagacctacatctgcaacgtgaaccacaagccctccaacaccaaggtggacaagaaggtggagcccaagtcctgcgacaagacccacacctgccctccctgccccgcccccgagctgctgggcggcccctccgtgttcctgttccctcctaagcccaaggacaccctgatgatctcccggacccccgaggtgacttgcgtggtggtggacgtgtcccacgaggaccccgaggtgaagttcaactggtacgtggacggcgtggaggtgcacaacgccaagaccaagccccgggaggagcagtacaactccacctaccgggtggtgtccgtgctgaccgtgctgcaccaggactggctgaacggcaaggagtacaagtgcaaggtgtccaacaaggccctgcccgcccccatcgagaagaccatctccaaggccaagggccagccccgggagccccaggtgtacaccctgcccccctcccgggaggagatgaccaagaaccaggtgtccctgacctgcctggtgaagggcttctacccctccgacatcgccgtggagtgggagtccaacggccagcccgagaacaactacaagaccaccccccccgtgctggactccgacggctccttcttcctgtactccaagctgaccgtggacaagtcccggtggcagcagggcaacgtgttctcctgctccgtgatgcacgaggccctgcacaaccactacacccagaagtccctgtccctgtcccccggcaag

SEQ ID NO: 108 - protein, 106 aa, synthetic construct
  REGION 1..106: note = Light Chain constant region
GQPKAAPSVTLFPPSSEELQANKATLVCLISDFYPGAVTVAWKADSSPVKAGVETTTPSKQSNNKYAASSYLSLTPEQWKSHRSYSCQVTHEGSTVEKTVAPAECS

SEQ ID NO: 109 - DNA, 330 bp, synthetic construct
  misc_feature 1..330: note = DNA encoding light chain variable region_BA6M11
  source 1..330: mol_type = other DNA
cagtccgtgctgacccagcccccctccgcctccggcacccccggccagcgggtgaccatctcctgctccggctcctcctccaacatcggctccaacgacgtgtcctggtaccagcagctgcccggcaccgcccccaagctgctgatctactacgaaaacaaccggccctccggcgtgcccgaccggttctccggctccaagtccggcacctccgcctccctggccatctccggcctgcggtccgaggacgaggccgactactactgcggcgcctgggacgactccctgtccggctacgtgttcggcggcggcaccaagctgaccgtgctg

SEQ ID NO: 110 - DNA, 318 bp, synthetic construct
  misc_feature 1..318: note = DNA encoding light chain constant region_BA6M11
  source 1..318: mol_type = other DNA
ggccagcccaaggccgccccctccgtgaccctgttccccccctcctccgaggagctgcaggccaacaaggccaccctggtgtgcctgatctccgacttctaccccggcgccgtgaccgtggcctggaaggccgactcctcccccgtgaaggccggcgtggagaccaccaccccctccaagcagtccaacaacaagtacgccgcctcctcctacctgtccctgacccccgagcagtggaagtcccaccggtcctactcctgccaggtgacccacgagggctccaccgtggagaagaccgtggcccccgccgagtgctcc

SEQ ID NO: 111 - protein, 216 aa, synthetic construct
  REGION 1..216: note = Light chain_BA6M11
QSVLTQPPSASGTPGQRVTISCSGSSSNIGSNDVSWYQQLPGTAPKLLIYYENNRPSGVPDRFSGSKSGTSASLAISGLRSEDEADYYCGAWDDSLSGYVFGGGTKLTVLGQPKAAPSVTLFPPSSEELQANKATLVCLISDFYPGAVTVAWKADSSPVKAGVETTTPSKQSNNKYAASSYLSLTPEQWKSHRSYSCQVTHEGSTVEKTVAPAECS

SEQ ID NO: 112 - protein, 451 aa, synthetic construct
  REGION 1..451: note = Heavy chain_BA6M11(WT)
EVQLLESGGGLVQPGGSLRLSCAASGFTFSNYDMSWVRQAPGKGLEWVSAIYHSGSSKYYADSVKGRFTISRDNSKNTLYLQMNSLRAEDTAVYYCARGGSGAWDTGFDYWGQGTLVTVSSASTKGPSVFPLAPSSKSTSGGTAALGCLVKDYFPEPVTVSWNSGALTSGVHTFPAVLQSSGLYSLSSVVTVPSSSLGTQTYICNVNHKPSNTKVDKKVEPKSCDKTHTCPPCPAPELLGGPSVFLFPPKPKDTLMISRTPEVTCVVVDVSHEDPEVKFNWYVDGVEVHNAKTKPREEQYNSTYRVVSVLTVLHQDWLNGKEYKCKVSNKALPAPIEKTISKAKGQPREPQVYTLPPSREEMTKNQVSLTCLVKGFYPSDIAVEWESNGQPENNYKTTPPVLDSDGSFFLYSKLTVDKSRWQQGNVFSCSVMHEALHNHYTQKSLSLSPGK

SEQ ID NO: 113 - protein, 18 aa, synthetic construct
  REGION 1..18: note = Linker1
GSGSGSGSGSGSGSGSGS

SEQ ID NO: 114 - protein, 20 aa, synthetic construct
  REGION 1..20: note = Linker2
GGGGSGGGGSGGGGSGGGGS

SEQ ID NO: 115 - protein, 720 aa, synthetic construct
  REGION 1..720: note = Full-length_Heavy chain BA6M11(WT)x1A10M12
EVQLLESGGGLVQPGGSLRLSCAASGFTFSNYDMSWVRQAPGKGLEWVSAIYHSGSSKYYADSVKGRFTISRDNSKNTLYLQMNSLRAEDTAVYYCARGGSGAWDTGFDYWGQGTLVTVSSASTKGPSVFPLAPSSKSTSGGTAALGCLVKDYFPEPVTVSWNSGALTSGVHTFPAVLQSSGLYSLSSVVTVPSSSLGTQTYICNVNHKPSNTKVDKKVEPKSCDKTHTCPPCPAPELLGGPSVFLFPPKPKDTLMISRTPEVTCVVVDVSHEDPEVKFNWYVDGVEVHNAKTKPREEQYNSTYRVVSVLTVLHQDWLNGKEYKCKVSNKALPAPIEKTISKAKGQPREPQVYTLPPSREEMTKNQVSLTCLVKGFYPSDIAVEWESNGQPENNYKTTPPVLDSDGSFFLYSKLTVDKSRWQQGNVFSCSVMHEALHNHYTQKSLSLSPGKGSGSGSGSGSGSGSGSGSQSVLTQPPSASGTPGQRVTISCSGSSSNIGNNYVTWYQQLPGTAPKLLIYADSHRPSGVPDRFSGSKSGTSASLAISGLRSEDEADYYCATWDYSLSGYVFGCGTKLTVLGGGGSGGGGSGGGGSGGGGSEVQLLESGGGLVQPGGSLRLSCAASGFTFSSYDMSWVRQAPGKCLEWVSWISYSGGSIYYADSVKGRFTISRDNSKNTLYLQMNSLRAEDTAVYYCARDAQRNSMREFDYWGQGTLVTVSS

SEQ ID NO: 116 - protein, 451 aa, synthetic construct
  REGION 1..451: note = Heavy chain_BA6M11(NA)
EVQLLESGGGLVQPGGSLRLSCAASGFTFSNYDMSWVRQAPGKGLEWVSAIYHSGSSKYYADSVKGRFTISRDNSKNTLYLQMNSLRAEDTAVYYCARGGSGAWDTGFDYWGQGTLVTVSSASTKGPSVFPLAPSSKSTSGGTAALGCLVKDYFPEPVTVSWNSGALTSGVHTFPAVLQSSGLYSLSSVVTVPSSSLGTQTYICNVNHKPSNTKVDKKVEPKSCDKTHTCPPCPAPELLGGPSVFLFPPKPKDTLMISRTPEVTCVVVDVSHEDPEVKFNWYVDGVEVHNAKTKPREEQYASTYRVVSVLTVLHQDWLNGKEYKCKVSNKALPAPIEKTISKAKGQPREPQVYTLPPSREEMTKNQVSLTCLVKGFYPSDIAVEWESNGQPENNYKTTPPVLDSDGSFFLYSKLTVDKSRWQQGNVFSCSVMHEALHNHYTQKSLSLSPGK

SEQ ID NO: 117 - protein, 720 aa, synthetic construct
  REGION 1..720: note = Full-length_Heavy chain BA6M11(NA)x1A10M12
EVQLLESGGGLVQPGGSLRLSCAASGFTFSNYDMSWVRQAPGKGLEWVSAIYHSGSSKYYADSVKGRFTISRDNSKNTLYLQMNSLRAEDTAVYYCARGGSGAWDTGFDYWGQGTLVTVSSASTKGPSVFPLAPSSKSTSGGTAALGCLVKDYFPEPVTVSWNSGALTSGVHTFPAVLQSSGLYSLSSVVTVPSSSLGTQTYICNVNHKPSNTKVDKKVEPKSCDKTHTCPPCPAPELLGGPSVFLFPPKPKDTLMISRTPEVTCVVVDVSHEDPEVKFNWYVDGVEVHNAKTKPREEQYASTYRVVSVLTVLHQDWLNGKEYKCKVSNKALPAPIEKTISKAKGQPREPQVYTLPPSREEMTKNQVSLTCLVKGFYPSDIAVEWESNGQPENNYKTTPPVLDSDGSFFLYSKLTVDKSRWQQGNVFSCSVMHEALHNHYTQKSLSLSPGKGSGSGSGSGSGSGSGSGSQSVLTQPPSASGTPGQRVTISCSGSSSNIGNNYVTWYQQLPGTAPKLLIYADSHRPSGVPDRFSGSKSGTSASLAISGLRSEDEADYYCATWDYSLSGYVFGCGTKLTVLGGGGSGGGGSGGGGSGGGGSEVQLLESGGGLVQPGGSLRLSCAASGFTFSSYDMSWVRQAPGKCLEWVSWISYSGGSIYYADSVKGRFTISRDNSKNTLYLQMNSLRAEDTAVYYCARDAQRNSMREFDYWGQGTLVTVSS

SEQ ID NO: 118 - DNA, 2160 bp, synthetic construct
  misc_feature 1..2160: note = DNA encoding heavy chain BA6M11(WT)x1A10M12
  source 1..2160: mol_type = other DNA
gaggtgcagctgctggagtccggcggcggcctggtgcagcccggcggctccctgcggctgtcctgcgccgcctccggcttcaccttctccaactacgacatgtcctgggtgcggcaggcccccggcaagggcctggagtgggtgtccgccatctaccactccggctcctccaagtactacgccgactccgtgaagggccggttcaccatctcccgggacaactccaagaacaccctgtacctgcagatgaactccctgcgggccgaggacaccgccgtgtactactgcgcccggggcggctccggcgcctgggacaccggcttcgactactggggccagggcaccctggtgaccgtgtcctctgcttctaccaagggaccctctgtgttccctctggctccttccagcaagtctacctctggtggaaccgctgctctgggctgcctggtcaaggattactttcctgagcctgtgacagtgtcctggaactctggtgctctgacctctggcgtgcacacctttccagctgtgctgcagtcctctggcctgtactctctgtcctctgtcgtgaccgtgccatcttctagcctgggcacccagacctacatctgcaacgtgaaccacaagccttccaacaccaaggtggacaagaaggtggaacccaagtcctgcgacaagacccacacctgtcctccatgtcctgctccagaactgctcggcggtccctccgttttcctgtttccacctaagcctaaggacaccctgatgatctctcggacccctgaagtgacctgcgtggtggtggatgtgtctcacgaggatcccgaagtgaagttcaattggtacgtggacggcgtggaagtgcacaacgccaagaccaagcctagagaggaacagtacaactccacctacagagtggtgtctgtgctgaccgtgctgcaccaggattggctgaacggcaaagagtacaagtgcaaggtgtccaacaaggccctgcctgctcctatcgaaaagaccatctccaaggctaagggccagcctcgggaacctcaagtgtacaccctgcctcctagcagagaagagatgaccaagaaccaggtgtccctgacctgcctggtcaagggcttctacccttccgatatcgccgtggaatgggagtccaatggccagcctgagaacaactacaagaccacacctcctgtgctggactccgacggctcattcttcctgtactccaagctgaccgtggacaagtccagatggcagcagggcaacgtgttctcctgctccgtgatgcacgaggccctgcacaatcactacacccagaagtccctgtctctgtcccctggcaaaggctccggatctggttctggatccggaagcggttctggcagcggatctggatctcagtccgtgctgactcagcctccttctgcttctggcacccctggccaaagagtgacaatctcttgctccggctcctcctccaacatcggcaacaactacgtgacctggtatcagcagctgcccggcacagctcccaaactgctgatctacgccgactctcacagaccttccggcgtgcccgatagattctccggctctaagtctggcacctctgccagcctggctatctccggcctgagatctgaggacgaggccgactactactgcgccacctgggattattccctgtccggctacgtgttcggctgcggcacaaaactgacagtgcttggcggcggaggatctggcggaggtggaagcggaggcggaggaagcggtggcggcggatctgaagttcagctgttggaaagtggcggaggcctggttcaacctggcggatctctgagactgtcttgtgccgcctccggctttaccttctcctcctacgacatgtcctgggtccgacaggctcctggcaagtgtctggaatgggtttcctggatctcctactccggcggctccatctactacgccgattccgtgaagggcagattcaccatcagccgggacaactccaagaacaccctgtacctgcagatgaactccctgagagccgaggacaccgccgtgtactactgtgctagagatgcccagcggaacagcatgagagagttcgactattggggccagggcaccctggtcacagtctcttct

SEQ ID NO: 119 - DNA, 648 bp, synthetic construct
  misc_feature 1..648: note = DNA encoding light chain BA6M11
  source 1..648: mol_type = other DNA
cagtccgtgctgacccagcccccctccgcctccggcacccccggccagcgggtgaccatctcctgctccggctcctcctccaacatcggctccaacgacgtgtcctggtaccagcagctgcccggcaccgcccccaagctgctgatctactacgaaaacaaccggccctccggcgtgcccgaccggttctccggctccaagtccggcacctccgcctccctggccatctccggcctgcggtccgaggacgaggccgactactactgcggcgcctgggacgactccctgtccggctacgtgttcggcggcggcaccaagctgaccgtgctgggccagcccaaggccgccccctccgtgaccctgttccccccctcctccgaggagctgcaggccaacaaggccaccctggtgtgcctgatctccgacttctaccccggcgccgtgaccgtggcctggaaggccgactcctcccccgtgaaggccggcgtggagaccaccaccccctccaagcagtccaacaacaagtacgccgcctcctcctacctgtccctgacccccgagcagtggaagtcccaccggtcctactcctgccaggtgacccacgagggctccaccgtggagaagaccgtggcccccgccgagtgctcc

SEQ ID NO: 120 - protein, 15 aa, synthetic construct
  REGION 1..15: note = Linker1
GGGGSGGGGSGGGGS

SEQ ID NO: 121 - protein, 712 aa, synthetic construct
  REGION 1..712: note = Full-length_Heavy chain BA6M11(WT)xB5
EVQLLESGGGLVQPGGSLRLSCAASGFTFSNYDMSWVRQAPGKGLEWVSAIYHSGSSKYYADSVKGRFTISRDNSKNTLYLQMNSLRAEDTAVYYCARGGSGAWDTGFDYWGQGTLVTVSSASTKGPSVFPLAPSSKSTSGGTAALGCLVKDYFPEPVTVSWNSGALTSGVHTFPAVLQSSGLYSLSSVVTVPSSSLGTQTYICNVNHKPSNTKVDKKVEPKSCDKTHTCPPCPAPELLGGPSVFLFPPKPKDTLMISRTPEVTCVVVDVSHEDPEVKFNWYVDGVEVHNAKTKPREEQYNSTYRVVSVLTVLHQDWLNGKEYKCKVSNKALPAPIEKTISKAKGQPREPQVYTLPPSREEMTKNQVSLTCLVKGFYPSDIAVEWESNGQPENNYKTTPPVLDSDGSFFLYSKLTVDKSRWQQGNVFSCSVMHEALHNHYTQKSLSLSPGKGGGGSGGGGSGGGGSQSVLTQPPSASGTPGQRVTISCSGSSSNIGSNAVSWYQQLPGTAPKLLIYYNSHRPSGVPDRFSGSKSGTSASLAISGLRSEDEADYYCGSWDASLNAYVFGCGTKLTVLGGGGSGGGGSGGGGSGGGGSEVQLLESGGGLVQPGGSLRLSCAASGFTFSDYAMSWVRQAPGKCLEWVSSISSGSGSIYYADSVKGRFTISRDNSKNTLYLQMNSLRAEDTAVYYCAKNLIPLDYWGQGTLVTVSS

SEQ ID NO: 122 - DNA, 2136 bp, synthetic construct
  misc_feature 1..2136: note = DNA encoding Heavy chain BA6M11(WT)x B5
  source 1..2136: mol_type = other DNA
gaagttcagctgctggaatctggcggcggattggttcaacctggcggctctctgagactgtcttgtgccgcttctggcttcaccttctccaactacgacatgtcctgggtccgacaggctcccggcaaaggattggaatgggtgtccgccatctaccactccggctcctctaagtactacgccgactccgtgaagggcagattcaccatctctcgggacaactccaagaacaccctgtacctgcagatgaactccctgagagccgaggacaccgccgtgtactattgtgccagaggcggatctggcgcctgggacaccggctttgattattggggacagggcaccctggtgaccgtgtcctccgcctccaccaagggcccctccgtgttccccctggccccctcctccaagtccacctccggcggcaccgccgccctgggctgcctggtgaaggactacttccccgagcccgtgaccgtgtcctggaactccggcgccctgacctccggcgtgcacaccttccccgccgtgctgcagtcctccggcctgtactccctgtcctccgtcgtgaccgtgccctcctcctccctgggcacccagacctacatctgcaacgtgaaccacaagccctccaacaccaaggtggacaagaaggtggagcccaagtcctgcgacaagacccacacctgccctccctgccccgcccccgagctgctgggcggcccctccgtgttcctgttccctcctaagcccaaggacaccctgatgatctcccggacccccgaggtgacttgcgtggtggtggacgtgtcccacgaggaccccgaggtgaagttcaactggtacgtggacggcgtggaggtgcacaacgccaagaccaagccccgggaggagcagtacaactccacctaccgggtggtgtccgtgctgaccgtgctgcaccaggactggctgaacggcaaggagtacaagtgcaaggtgtccaacaaggccctgcccgcccccatcgagaagaccatctccaaggccaagggccagccccgggagccccaggtgtacaccctgcctcctagcagagaagagatgaccaagaaccaggtgtccctgacctgcctggtcaagggcttctacccttccgatatcgccgtggaatgggagtccaatggccagcctgagaacaactacaagaccacacctcctgtgctggactccgacggctcattcttcctgtactccaagctgaccgtggacaagtccagatggcagcagggcaacgtgttctcctgctccgtgatgcacgaggccctgcacaatcactacacccagaagtccctgtctctgtcccctggaaaaggcggcggaggatctggcggaggtggaagcggaggcggtggatctcagtctgttctgacccagcctccttccgcttctggcacacctggacagagagtgaccatctcttgctccggctcctcctccaacatcggctctaatgccgtgtcctggtatcagcagctgcctggcacagctcccaaactgctgatctactacaactcccaccggccttccggcgtgcccgatagattttccggctctaagtccggcacctctgccagcctggctatctctggcctgagatctgaggacgaggccgactactactgcggctcttgggatgcctctctgaacgcctacgtgttcggctgtggcacaaagctgacagtgcttggaggtggtggtagtggtggtggcggttcaggtggcggaggaagcggcggaggcggatctgaagttcagctgttggaatctggcggcggactggttcaacctggcggatctctgagactgtcttgtgccgcctctggcttcaccttctccgactacgctatgtcttgggtccgacaggcccctggcaagtgtctggaatgggtttcctccatctcctccggcagcggctctatctactacgccgactctgtgaagggcagattcaccatcagccgggacaactccaagaacaccctgtacctgcagatgaactccctgagagccgaggacaccgccgtgtactactgtgccaagaatctgatccctctggactactggggccagggcacactggttacagtgtcctct

SEQ ID NO: 123 - DNA, 648 bp, synthetic construct; identical to SEQ ID NO: 119
  misc_feature 1..648: note = DNA encoding Light chain BA6M11
  source 1..648: mol_type = other DNA

SEQ ID NO: 124 - protein, 216 aa, synthetic construct
  REGION 1..216: note = Light chain BA6
QSVLTQPPSASGTPGQRVTISCSGSSSNIGSNDVSWYQQLPGTAPKLLIYYDNNRPSGVPDRFSGSKSGTSASLAISGLRSEDEADYYCGAWDDSLSGYVFGGGTKLTVLGQPKAAPSVTLFPPSSEELQANKATLVCLISDFYPGAVTVAWKADSSPVKAGVETTTPSKQSNNKYAASSYLSLTPEQWKSHRSYSCQVTHEGSTVEKTVAPAECS

SEQ ID NO: 125 - protein, 720 aa, synthetic construct
  REGION 1..720: note = Heavy chain BA6x1A10M12
EVQLLESGGGLVQPGGSLRLSCAASGFTFSNYDMSWVRQAPGKGLEWVSAIYHSGSSKYYADSVKGRFTISRDNSKNTLYLQMNSLRAEDTAVYYCARGGNGAWDTGFDYWGQGTLVTVSSASTKGPSVFPLAPSSKSTSGGTAALGCLVKDYFPEPVTVSWNSGALTSGVHTFPAVLQSSGLYSLSSVVTVPSSSLGTQTYICNVNHKPSNTKVDKKVEPKSCDKTHTCPPCPAPELLGGPSVFLFPPKPKDTLMISRTPEVTCVVVDVSHEDPEVKFNWYVDGVEVHNAKTKPREEQYASTYRVVSVLTVLHQDWLNGKEYKCKVSNKALPAPIEKTISKAKGQPREPQVYTLPPSREEMTKNQVSLTCLVKGFYPSDIAVEWESNGQPENNYKTTPPVLDSDGSFFLYSKLTVDKSRWQQGNVFSCSVMHEALHNHYTQKSLSLSPGKGSGSGSGSGSGSGSGSGSQSVLTQPPSASGTPGQRVTISCSGSSSNIGNNYVTWYQQLPGTAPKLLIYADSHRPSGVPDRFSGSKSGTSASLAISGLRSEDEADYYCATWDYSLSGYVFGCGTKLTVLGGGGSGGGGSGGGGSGGGGSEVQLLESGGGLVQPGGSLRLSCAASGFTFSSYDMSWVRQAPGKCLEWVSWISYSGGSIYYADSVKGRFTISRDNSKNTLYLQMNSLRAEDTAVYYCARDAQRNSMREFDYWGQGTLVTVSS

SEQ ID NO: 126 - protein, 110 aa, synthetic construct
  REGION 1..110: note = light chain variable region_anti-ROR1 antibody (scFv)
QSVLTQPPSASGTPGQRVTISCSGSSSNIGSNDVSWYQQLPGTAPKLLIYYENNRPSGVPDRFSGSKSGTSASLAISGLRSEDEADYYCGAWDDSLSGYVFGCGTKLTVL

SEQ ID NO: 127 - protein, 121 aa, synthetic construct
  REGION 1..121: note = heavy chain variable region_anti-ROR1 antibody (scFv)
EVQLLESGGGLVQPGGSLRLSCAASGFTFSNYDMSWVRQAPGKCLEWVSAIYHSGSSKYYADSVKGRFTISRDNSKNTLYLQMNSLRAEDTAVYYCARGGSGAWDTGFDYWGQGTLVTVSS